European Patent Specification EP 4 114 420 B1, published June 3, 2026. Title: USE OF COPROCOCCUS BACTERIA FOR THE TREATMENT OF METABOLIC SYNDROME AND INFLAMMATORY BOWEL DISEASES. Applicant: Institut national de recherche pour l'agriculture, l'alimentation et l'environnement ASSISTANCE PUBLIQUE- HÔPITAUX DE PARIS Sorbonne Université INSTITUT NATIONAL DE LA SANTÉ ET DE LA RECHERCHE MÉDICALE. The sequence listing filed with the application follows.

SEQUENCE LISTING (6 sequences)

SEQ ID NO: 1 - DNA, 22 bp, Artificial Sequence
  Primer Reg3gamma
ttcctgtcctccatgatcaaaa

SEQ ID NO: 2 - DNA, 21 bp, Artificial Sequence
  Primer Reg3gamma
catccacctctgttgggttca

SEQ ID NO: 3 - DNA, 21 bp, Artificial Sequence
  primer reg3beta
atgctgctctcctgcctgatg

SEQ ID NO: 4 - DNA, 24 bp, Artificial Sequence
  primer Reg3beta
ctaatgcgtgcggagggtatattc

SEQ ID NO: 5 - DNA, 20 bp, Artificial Sequence
  Primer AhRR
ggagtctctcaatggcttcg

SEQ ID NO: 6 - DNA, 20 bp, Artificial Sequence
  Primer AhRR
ccgagtactctgagggcaag